European Patent Application EP 4 461 369 A2, published November 13, 2024. Title: AEROSOLIZED COMPOSITIONS COMPRISING MITOCHONDRIA AND METHODS OF USE THEREOF. Applicant: Children's Medical Center Corporation. Application EP. The sequence listing filed with the application follows.

SEQUENCE LISTING (4 sequences)

SEQ ID NO: 1 - DNA, 20 bp, synthetic construct
  misc_feature 1..20: note = Primer for mouse mMitoF1
  source 1..20: mol_type = other DNA
ctagaaaccccgaaaccaaa

SEQ ID NO: 2 - DNA, 20 bp, synthetic construct
  misc_feature 1..20: note = Primer for mouse mMitoR1
  source 1..20: mol_type = other DNA
ccagctatcaccaagctcgt

SEQ ID NO: 3 - DNA, 20 bp, synthetic construct
  misc_feature 1..20: note = Primer for mB2MR1
  source 1..20: mol_type = other DNA
atgggaagccgaacatactg

SEQ ID NO: 4 - DNA, 20 bp, synthetic construct
  misc_feature 1..20: note = Primer for mB2MR1
  source 1..20: mol_type = other DNA
cagtctcagtgggggtgaat